European Patent Specification EP 3 895 724 B1, published June 25, 2025. Title: EXTENDED RELEASE OF NEUREGULIN FOR TREATING HEART FAILURE. Applicant: Zensun (Shanghai) Science and Technology, Co., Ltd. Application Divisional application based on EP 19186339.8. The sequence listing filed with the application follows.

SEQUENCE LISTING (5 sequences)

SEQ ID NO: 1 - protein, 61 aa, Unknown
  Description of Unknown: Unknown neuregulin sequence
SHLVKCAEKEKTFCVNGGECFMVKDLSNPSRYLCKCPNEFTGDRCQNYVMASFYKAEELYQ

SEQ ID NO: 2 - protein, 50 aa, Unknown
  Description of Unknown: Unknown neuregulin sequence
SHLVKCAEKEKTFCVNGGECFMVKDLSNPSRYLCKCPNEFTGDRCQNYVM

SEQ ID NO: 3 - protein, 64 aa, Unknown
  Description of Unknown: Unknown neuregulin sequence
SHLVKCAEKEKTFCVNGGECFMVKDLSNPSRYLCKCPNEFTGDRCQNYVMASFYKAEELYQKRV

SEQ ID NO: 4 - protein, 23 aa, Unknown
  Description of Unknown: Unknown neuregulin sequence
AEKEKTFCVNGGECFMVKDLSNP

SEQ ID NO: 5 - protein, 68 aa, Unknown
  Description of Unknown: Unknown neuregulin sequence
SHLVKCAEKEKTFCVNGGECFMVKDLSNPSRYLCKCPNEFTGDRCQNYVMASFYKAEELYQKRVLTIT